European Patent Application EP 4 538 394 A2, published April 16, 2025. Title: COMPOSITIONS AND METHODS FOR AMPLIFYING OR DETECTING VARICELLA-ZOSTER VIRUS. Applicant: Carvallo Pinto, Marcella Alejandra. Application US PCT/US2019/053943, filed October 1, 2019. The sequence listing filed with the application follows.

SEQUENCE LISTING (42 sequences)

SEQ ID NO: 1 - DNA, 20 bp, synthetic construct
  misc_feature 1..20: note = Synthetic oligonucleotide
  source 1..20: mol_type = other DNA
ttgcttccccacaccgttta

SEQ ID NO: 2 - DNA, 23 bp, synthetic construct
  misc_feature 1..23: note = Synthetic oligonucleotide
  source 1..23: mol_type = other DNA
gcggtattctgtaaaggatctcc

SEQ ID NO: 3 - DNA, 22 bp, synthetic construct
  misc_feature 1..22: note = Synthetic oligonucleotide
  source 1..22: mol_type = other DNA
ctacttttatcgcggcttgttg

SEQ ID NO: 4 - DNA, 21 bp, synthetic construct
  misc_feature 1..21: note = Synthetic oligonucleotide
  source 1..21: mol_type = other DNA
ccaaaactaacaaagccggga

SEQ ID NO: 5 - DNA, 21 bp, synthetic construct
  misc_feature 1..21: note = Synthetic oligonucleotide
  source 1..21: mol_type = other DNA
cttgcttcgtcgctgaaatcc

SEQ ID NO: 6 - DNA, 21 bp, synthetic construct
  misc_feature 1..21: note = Synthetic oligonucleotide
  source 1..21: mol_type = other DNA
gtaaaacgcacatggctgtgt

SEQ ID NO: 7 - DNA, 20 bp, synthetic construct
  misc_feature 1..20: note = Synthetic oligonucleotide
  source 1..20: mol_type = other DNA
gggcctgaattatacttgga

SEQ ID NO: 8 - DNA, 25 bp, synthetic construct
  misc_feature 1..25: note = Synthetic oligonucleotide
  source 1..25: mol_type = other DNA
ggatctccacgtagcaaagctacac

SEQ ID NO: 9 - DNA, 26 bp, synthetic construct
  misc_feature 1..26: note = Synthetic oligonucleotide
  source 1..26: mol_type = other DNA
gctacactttttgcatcagcctccac

SEQ ID NO: 10 - DNA, 23 bp, synthetic construct
  misc_feature 1..23: note = Synthetic oligonucleotide
  source 1..23: mol_type = other DNA
gcgcgcatacccggaagttcttc

SEQ ID NO: 11 - DNA, 23 bp, synthetic construct
  misc_feature 1..23: note = Synthetic oligonucleotide
  source 1..23: mol_type = other DNA
cgagtggtagcgtctacccgacc

SEQ ID NO: 12 - DNA, 23 bp, synthetic construct
  misc_feature 1..23: note = Synthetic oligonucleotide
  source 1..23: mol_type = other DNA
ggtcgggtagacgctaccactcg

SEQ ID NO: 13 - DNA, 27 bp, synthetic construct
  misc_feature 1..27: note = Synthetic oligonucleotide
  source 1..27: mol_type = other DNA
gccaacatcccatatcttaaacagacc

SEQ ID NO: 14 - DNA, 26 bp, synthetic construct
  misc_feature 1..26: note = Synthetic oligonucleotide
  source 1..26: mol_type = other DNA
catctgtgcgctcaataacctcaacg

SEQ ID NO: 15 - DNA, 24 bp, synthetic construct
  misc_feature 1..24: note = Synthetic oligonucleotide
  source 1..24: mol_type = other DNA
tgcaaaatccaatacgaccaccgg

SEQ ID NO: 16 - DNA, 20 bp, synthetic construct
  misc_feature 1..20: note = Synthetic oligonucleotide
  source 1..20: mol_type = other DNA
cgttcgagaacgcatccctt

SEQ ID NO: 17 - DNA, 22 bp, synthetic construct
  misc_feature 1..22: note = Synthetic oligonucleotide
  source 1..22: mol_type = other DNA
cgagaacgcatcccttatgtta

SEQ ID NO: 18 - DNA, 19 bp, synthetic construct
  misc_feature 1..19: note = Synthetic oligonucleotide
  source 1..19: mol_type = other DNA
ctatgcgcaaggctattag

SEQ ID NO: 19 - DNA, 23 bp, synthetic construct
  misc_feature 1..23: note = Synthetic oligonucleotide
  source 1..23: mol_type = other DNA
gtgataactttcacccggagttg

SEQ ID NO: 20 - DNA, 21 bp, synthetic construct
  misc_feature 1..21: note = Synthetic oligonucleotide
  source 1..21: mol_type = other DNA
gggcgtttattatggagaaac

SEQ ID NO: 21 - DNA, 19 bp, synthetic construct
  misc_feature 1..19: note = Synthetic oligonucleotide
  source 1..19: mol_type = other DNA
ggagacaagaacgcttttc

SEQ ID NO: 22 - DNA, 21 bp, synthetic construct
  misc_feature 1..21: note = Synthetic oligonucleotide
  source 1..21: mol_type = other DNA
ggatataaaggagccagggtt

SEQ ID NO: 23 - DNA, 20 bp, synthetic construct
  misc_feature 1..20: note = Synthetic oligonucleotide
  source 1..20: mol_type = other DNA
tccaaagcatggcatactac

SEQ ID NO: 24 - DNA, 20 bp, synthetic construct
  misc_feature 1..20: note = Synthetic oligonucleotide
  source 1..20: mol_type = other DNA
ggcatactaccaatgacacg

SEQ ID NO: 25 - DNA, 22 bp, synthetic construct
  misc_feature 1..22: note = Synthetic oligonucleotide
  source 1..22: mol_type = other DNA
gaaaacactaatcattcaccac

SEQ ID NO: 26 - DNA, 23 bp, synthetic construct
  misc_feature 1..23: note = Synthetic oligonucleotide
  source 1..23: mol_type = other DNA
caatagttagtttaaatgggtcc

SEQ ID NO: 27 - DNA, 23 bp, synthetic construct
  misc_feature 1..23: note = Synthetic oligonucleotide
  source 1..23: mol_type = other DNA
ctagactacagtgaaattcaacg

SEQ ID NO: 28 - DNA, 23 bp, synthetic construct
  misc_feature 1..23: note = Synthetic oligonucleotide
  source 1..23: mol_type = other DNA
atgatgcaattcaccgacgtgcc

SEQ ID NO: 29 - DNA, 22 bp, synthetic construct
  misc_feature 1..22: note = Synthetic oligonucleotide
  source 1..22: mol_type = other DNA
agatcccgacgaagcgtgccag

SEQ ID NO: 30 - DNA, 22 bp, synthetic construct
  misc_feature 1..22: note = Synthetic oligonucleotide
  source 1..22: mol_type = other DNA
ctggcacgcttcgtcgggatct

SEQ ID NO: 31 - DNA, 24 bp, synthetic construct
  misc_feature 1..24: note = Synthetic oligonucleotide
  source 1..24: mol_type = other DNA
ccatgcgtggctaatcacaagcga

SEQ ID NO: 32 - DNA, 27 bp, synthetic construct
  misc_feature 1..27: note = Synthetic oligonucleotide
  source 1..27: mol_type = other DNA
ggttgtgcaatatgatagcggaacggc

SEQ ID NO: 33 - DNA, 27 bp, synthetic construct
  misc_feature 1..27: note = Synthetic oligonucleotide
  source 1..27: mol_type = other DNA
gccgttccgctatcatattgcacaacc

SEQ ID NO: 34 - DNA, 20 bp, synthetic construct
  misc_feature 1..20: note = Synthetic oligonucleotide
  source 1..20: mol_type = other DNA
gatctggcttcaacttcctc

SEQ ID NO: 35 - DNA, 21 bp, synthetic construct
  misc_feature 1..21: note = Synthetic oligonucleotide
  source 1..21: mol_type = other DNA
tgttctattggcacgcaactc

SEQ ID NO: 36 - DNA, 22 bp, synthetic construct
  misc_feature 1..22: note = Synthetic oligonucleotide
  source 1..22: mol_type = other DNA
cataatatacgtagtgatgccc

SEQ ID NO: 37 - DNA, 20 bp, synthetic construct
  misc_feature 1..20: note = Synthetic oligonucleotide
  source 1..20: mol_type = other DNA
gtccctggaaaaactgagcc

SEQ ID NO: 38 - DNA, 3610 bp, synthetic construct
  misc_feature 1..3610: note = Varicella-Zoster Virus partial sequence
  source 1..3610: mol_type = other DNA
tttactgtaaaatgtgtgaccttaactttgatggagaattgcttttggaatacaaaagactctacgcattatttgatgactttgttcctcctcggtgatttcagcttcagtgttcattttattatcccagcacggggcgtgtatacaaacaaagcctgccgcctgcaagcggtttagcattttaacgttaacaactcgtgtctctggaataaaacgttttaaaagccgttctgtgagtttagtgtcgtttccaaataacgccttaaaagttacactcgccgtcccaatgagatgagaaaaataatagtcaatgtttaaagacagcccgtgtgatgttacgtgaatgggatcttccgctaagtcagatattattaacttacgctttgcttccccacaccgtttacctgcggtattctgtaaaggatctccacgtagcaaagctacactttttgcatcagcctccacttcgtctgtgggggccacaataacataagggatgcgttctcgaacgtttgggatttgaccctgtctcattactaatttataatatactgttaagtgagccaagcgacggtttatgtaggcggatggtggacgactaagctcggccgtcataacaaacttattaatatccaatttgggtgatgtaatctggcgatgtgcatctgcaattatgcgtccaaacccggccatcccagacggcatggcccgtctattccattcagcaatggaaacacacgacgcctccgccgcagcacgcgagacggtgtcgtcatataacaacagttctacaagtttgcgggcataatcgttaataaattgacagttgttttttctaaccaagtcgactcccttcattaaaacctttccgccgtaaattaccccaatgtactttttctttgttataagcaaaagttttataaaagttttttcacactccaactttataggaggacaaaacagagccgttgaaattatatgtgccattttctcgccgattttagctatcccctcaacactaacacccttgaatcggataaacacagaatccgtatctccatatataacctttacctcgtacgctttttgggagagaacgctactttcaatgtctggaaacgctgtaataaaacgttcaaatgcggcccagttattatgaatataatctctggtacttaataacatttgacggccaattgtagtgacagtggccgctacgtataaacatggcagaaatccctgcgcaactccagtaaaaccgtacacggaattacaaactacttttatcgcggcttgttgtttgtctaataacactgcttcatctgaagaacttccgggtatgcgcgctctaatagccttgcgcatagccaaccagtcttttaaaagaacacccagcagactttctcgaacgttagagcgcacaaaaaaaagacgttttcctccaactgtaaaggtggcataatcggatggattcaaacgtttaaccgtctcaaaatttaacgttagcgtggtaaaacataagttatgggcctgaattatacttggatataaacttgcaaaatccaatacgaccaccggatcgatataaaatcccgtatcagggtcaaaaaccctggctcctttatatcctacatttcgcccacttgacgtaccagtgggagaaacgctctcgtcttcatccatctcttcctcaacatccccgacatcgggaataacatccttatattcaaaagtagctgggtatcccccatcgggtaaaataaatcctcgagacgaagccagtcctaataaacaggtgtaaatcctaacctgctgtccgtcgtaaatagccttggttaaagtaattctagctagccttgcaaccgcggataactcaaggtgtggtaaatatttaaaaaacagtttccccacaagagccgagtcttgtatacaatattcaccaataattcctcgtgtattcggtccactagcgtaatatcccggaatgtctttgtagggcaaatctctcttggactcatttagagcttcacgtgcaaccgaatctaatttataactcgagagttttaatttttcagttgcaattgcatacatatccagagatatgagaccgttgatctttaccttgcttcgtcgctgaaatccggatttgccaacatcccatatcttaaacagacccccacggtttatactgccataaccatcaagcttgagactgtatatagaattaagtttctccataataaacgcccaatcaaaattaacaatgttataacctgtggcaaactcgggagcgtactgttttacgagggtcataaatgcaattaatagctcgaattcactatcaaactccagcacagtcggctccggtaaccccgcgtccttcatttcttgtacatacctttgtggtaagtcacaagagccaagggaaaacagtaaaatgtgttctaaagactgtcgagggattgaatataatagacaagaaatttggattacaagatcctccagatgtgttgcatcgggaaacgccagctcattagatcctcctgatttacattcaatatcgaaacataacaacttgtagtcaggccatgagtcatcgtttggtatagcctgcagattatccgacatgcagtcaatttcaacgtcgcttaacgttaattggcgacttgccggtcgaactcgaacacgttccccatcaactccaggttttagttgataccaaccaaaactaacaaagccgggattatccattagaaaacgagtggtagcgtctacccgaccttcatactttttcaactccgggtgaaagttatcacaaagataatttgtaaatttagatgagggagaatacaccctgtaaaacgcacatggctgtgtatcgtagtaataaacatctgtgcgctcaataacctcaacgcgaaagctttctggagatgcgcttttaaacgaggtaccatgaaaagcgttcttgtctccatttaacgttgcatcattttgtgttatcatagaactgcgtaaacactcggcaagtaatacagataactcgctaccggaacgtatgccacaagcggtatccacctcggctttgtttatataaaaatattgacagatgccgtatacatgaactgccaccctttttccacatcgggacatgccaagtaaagtaataacggtaccaagcggtcgtgttgcagttgcaaaccgggatacatctccattagacgcggcttctgttgtttcgacaatatcatatacatggaatgtgttaaagcgggggtcaaacttatccccacgaaagtcgatttccccccaaatattcacgcgtctaggccaggggctggaacaacgaaaatccagaatcggaacttcttttccattacagtaaactttaggcggtcgactaagtgtaccgacgtgaaccccctttcgttcttccatgggcacatcttcatctaaacatttaggggccaaaaattgaaacgatgacatggtagttttgtaactatgaagaaattctctgttactaccgcgcccggttcttgggttatatttaatccctgatgcttgggttaaaaagggattacaaaaccccgttctgatcgccatttta

SEQ ID NO: 39 - DNA, 2830 bp, synthetic construct
  misc_feature 1..2830: note = Varicella-Zoster Virus partial sequence
  source 1..2830: mol_type = other DNA
atgtccccttgtggctattattcaaagtggagaaacagggatcgaccagaataccgtcgtaatctacgattcagacgttttttctcttctatacaccctaatgcagcggctggctccggattcaacggacccggcgttttcataacctccgttacgggggtgtggttatgctttttatgcatattttctatgtttgttacggcggttgtgtcggtctctccaagctcgttttatgagagtttacaagtagagcccacacaatcagaagatataacccggtctgctcatctgggcgatggtgatgaaatcagagaagctatacacaagtcccaggacgccgaaacaaaacccacgttttacgtctgcccaccgccaacaggctccacaatcgtacgattagaaccaactcggacatgtccggattatcaccttggtaaaaactttacagagggtattgctgttgtttataaagaaaacattgcagcgtacaagtttaaggcgacggtatattacaaagatgttatcgttagcacggcgtgggccggaagttcttatacgcaaattactaatagatatgcggatagggtaccaattcccgtttcagagatcacggacaccattgataagtttggcaagtgttcttctaaagcaacgtacgtacgaaataaccacaaagttgaagcctttaatgaggataaaaatccacaggatatgcctctaatcgcatcaaaatataattctgtgggatccaaagcatggcatactaccaatgacacgtacatggttgccggaacccccggaacatataggacgggcacgtcggtgaattgcatcattgaggaagttgaagccagatcaatattcccttatgatagttttggactttccacgggagatataatatacatgtccccgttttttggcctacgggatggtgcatacagagaacattccaattatgcaatggatcgttttcaccagtttgagggttatagacaaagggatcttgacactagagcattactggaacctgcagcgcggaactttttagtcacgcctcatttaacggttggttggaactggaagccaaaacgaacggaagtttgttcgcttgtcaagtggcgtgaggttgaagacgtagttcgcgatgagtatgcacacaattttcgctttacaatgaaaacactttctaccacgtttataagtgaaacaaacgagtttaatcttaaccaaatccatctcagtcaatgtgtaaaggaggaagcccgggctattattaaccggatctatacaaccagatacaactcatctcatgttagaaccggggatatccagacctaccttgccagaggggggtttgttgtggtgtttcaacccctgctgagcaattccctcgcccgtctctatctccaagaattggtccgtgaaaacactaatcattcaccacaaaaacacccgactcgaaataccagatcccgacgaagcgtgccagttgagttgcgtgccaatagaacaataacaaccacctcatcggtggaatttgctatgctccagtttacatatgaccacattcaagagcatgttaatgaaatgttggcacgtatctcctcgtcgtggtgccagctacaaaatcgcgaacgcgccctttggagcggactatttccaattaacccaagtgctttagcgagcaccattttggatcaacgtgttaaagctcgtattctcggcgacgttatctccgtttctaattgtccagaactgggatcagatacacgcattatacttcaaaactctatgagggtatctggtagtactacgcgttgttatagccgtcctttaatttcaatagttagtttaaatgggtccgggacggtggagggccagcttggaacagataacgagttaattatgtccagagatctgttagaaccatgcgtggctaatcacaagcgatattttctatttgggcatcactacgtatattatgaggattatcgttacgtccgtgaaatcgcagtccatgatgtgggaatgattagcacttacgtagatttaaacttaacacttcttaaagatagagagtttatgccgctgcaagtatatacaagagacgagctgcgggatacaggattactagactacagtgaaattcaacgccgaaatcaaatgcattcgctgcgtttttatgacatagacaaggttgtgcaatatgatagcggaacggccattatgcagggcatggctcagtttttccagggacttgggaccgcgggccaggccgttggacatgtggttcttggggccacgggagcgctgctttccaccgtacacggatttaccacgtttttatctaacccatttggggcattggccgtgggattattggttttggcgggactggtagcggccttttttgcgtaccggtacgtgcttaaacttaaaacaagcccgatgaaggcattatatccactcacaaccaaggggttaaaacagttaccggaaggaatggatccctttgccgagaaacccaacgctactgataccccaatagaagaaattggcgactcacaaaacactgaaccgtcggtaaatagcgggtttgatcccgataaatttcgagaagcccaggaaatgattaaatatatgacgttagtatctgcggctgagcgccaagaatctaaagcccgcaaaaaaaataagactagcgcccttttaacttcacgtcttaccggccttgctttacgaaatcgccgaggatactcccgtgttcgcaccgagaatgtaacgggggtgtaaatagccagggggtttgttttaatttattaataaa

SEQ ID NO: 40 - DNA, 20 bp, synthetic construct
  misc_feature 1..20: note = synthetic oligonucleotide
  source 1..20: mol_type = other DNA
atggtcaattagagacaaag

SEQ ID NO: 41 - DNA, 20 bp, synthetic construct
  misc_feature 1..20: note = synthetic oligonucleotide
  source 1..20: mol_type = other DNA
cgttcactattggtctctgc

SEQ ID NO: 42 - DNA, 26 bp, synthetic construct
  misc_feature 1..26: note = synthetic oligonucleotide
  source 1..26: mol_type = other DNA
cggaatcacaagtcaatcatcgcgca